European Patent Specification EP 3 431 600 B1, published February 14, 2024. Title: FAD2 PERFORMANCE LOCI AND CORRESPONDING TARGET SITE SPECIFIC BINDING PROTEINS CAPABLE OF INDUCING TARGETED BREAKS. Applicant: DOW AGROSCIENCES LLC. Application PCT/US2013/058299. The sequence listing filed with the application follows.

SEQUENCE LISTING (130 sequences)

SEQ ID NO: 1 - DNA, 22 bp, Artificial Sequence
  Description of Artificial Sequence: Synthetic primer
caagggttccaaacacaaagcc

SEQ ID NO: 2 - DNA, 22 bp, Artificial Sequence
  Description of Artificial Sequence: Synthetic primer
catcaatacttgttcctgtacc

SEQ ID NO: 3 - DNA, 23 bp, Artificial Sequence
  Description of Artificial Sequence: Synthetic primer
gaagaagcctctctcaagggttc

SEQ ID NO: 4 - DNA, 1100 bp, Glycine max
ggaagaagcctctctcaagggttccaaacacaaagccaccattcactgttggccaactcaagaaagcaattccaccacactgctttcagcgctccctcctcacttcattctcctatgttgtttatgacctttcatttgccttcattttctacattgccaccacctacttccacctccttcctcaacccttttccctcattgcatggccaatctattgggttctccaaggttgccttctcactggtgtgtgggtgattgctcacgagtgtggtcaccatgccttcagcaagtaccaatgggttgatgatgttgtgggtttgacccttcactcaacacttttagtcccttatttctcatggaaaataagccatcgccgccatcactccaacacaggttcccttgaccgtgatgaagtgtttgtcccaaaaccaaaatccaaagttgcatggttttccaagtacttaaacaaccctctaggaagggctgtttctcttctcgtcacactcacaatagggtggcctatgtatttagccttcaatgtctctggtagaccctatgatagttttgcaagccactaccacccttatgctcccatatattctaaccgtgagaggcttctgatctatgtctctgatgttgctttgttttctgtgacttactctctctaccgtgttgcaaccctgaaagggttggtttggctgctatgtgtttatggggtgcctttgctcattgtgaacggttttcttgtgactatcacatatttgcagcacacacactttgccttgcctcattacgattcatcagaatgggactggctgaagggagctttggcaactatggacagagattatgggattctgaacaaggtgtttcatcacataactgatactcatgtggctcaccatctcttctctacaatgccacattaccatgcaatggaggcaaccaatgcaatcaagccaatattgggtgagtactaccaatttgatgacacaccattttacaaggcactgtggagagaagcgagagagtgcctctatgtggagccagatgaaggaacatccgagaagggcgtgtattggtacaggaacaagtattga

SEQ ID NO: 5 - DNA, 1100 bp, Glycine max; identical to SEQ ID NO: 4

SEQ ID NO: 6 - DNA, 1100 bp, Glycine max; identical to SEQ ID NO: 4

SEQ ID NO: 7 - DNA, 1100 bp, Glycine max; identical to SEQ ID NO: 4

SEQ ID NO: 8 - DNA, 1100 bp, Glycine max; identical to SEQ ID NO: 4

SEQ ID NO: 9 - DNA, 1101 bp, Glycine max
cagaagaagcctctctcaagggttccaaacacaaagccaccattcactgttggccaactcaagaaagccattccaccgcactgctttcagcgttccctcctcacttcattgtcctatgttgtttatgacctttcattggctttcattttctacattgccaccacctacttccacctcctccctcaccccttttccctcattgcatggccaatctattgggttctccaaggttgcattcttactggcgtgtgggtgattgctcacgagtgtggtcaccatgccttcagcaagtacccatgggttgatgatgttatgggtttgaccgttcactcagcacttttagtcccttatttctcatggaaaataagccatcgccgccaccactccaacacgggttcccttgaccgtgatgaagtgtttgtcccaaaaccaaaatccaaagttgcatggtacaccaagtacctgaacaaccctctaggaagggctgcttctcttctcatcacactcacaatagggtggcctttgtatttagccttcaatgtctctggcagaccctatgatggttttgctagccactaccacccttatgctcccatatattcaaatcgtgagaggcttttgatctatgtctctgatgttgctttgttttctgtgacttacttgctctaccgtgttgcaactatgaaagggttggtttggctgctatgtgtttatggggtgccattgctcattgtgaacggttttcttgtgaccatcacatatctgcagcacacacactatgccttgcctcactatgattcatcagaatgggattggctgaggggtgctttggcaactatggacagagattatggaattctgaacaaggtgtttcaccacataactgatactcatgtggctcaccatcttttctctacaatgccacattaccatgcaacggaggcaaccaatgcaatgaagccaatattgggtgagtactaccgatttgatgacacaccattttacaaggcactgtggagagaagcaagagagtgcctctatgtggagccagatgaaggaacatccgagaagggcgtgtattggtacaggaacaagtattga

SEQ ID NO: 10 - DNA, 1101 bp, Glycine max; identical to SEQ ID NO: 9

SEQ ID NO: 11 - DNA, 1101 bp, Glycine max
cagaagaagcctctctcaagggttccaaacacaaagccaccattcactgttggccaactcaagaaagccattccaccgcactgctttcagcgttccctcctcacttcattgtcctatgttgtttatgacctttcattggctttcattttctacattgccaccacctacttccacctcctccctcacccctttttcctcattgcatggccaatctattgggttctccaaggttgcattcttactggcgtgtgggtgattgctcacgagtgtggtcaccatgccttcagcaagtacccatgggttgatgatgttgtgggtttgaccgttcactcagcacttttagtcccttatttctcatggaaaataagccatcgccgccaccactccaacacgggttcccttgaccgtgatgaagtgtttgtcccaaaaccaaaatccaaagttgcatggtacaccaagtacctgaacaaccctctaggaagggctgcttctcttctcatcacactcacaatagggtggcctttgtatttagccttcaatgtctctggcagaccctatgatggttttgctagccactaccacccttatgctcctatatattcaaaccgtgagaggcttctgatctatgtctctgatgttgctttgttttctgtgacttacttgctctaccgtgttgcaactatgaaagggttggtttggctgctatgtgtttatggggtgccattgctcattgtgaacggttttcttgtgaccatcacatatctgcagcacacacactatgccttgcctcactatgattcatcagaatgggattggctgaggggtgctttggcaactatggacagagattatgggattctgaacaaggtgtttcaccacataactgatactcatgtggctcaccatcttttctctacaatgccacattaccatgcaacggaggcaaccaatgcaatgaagccaatattgggtgagtactaccgatttgatgacacaccattttacaaggcactgtggagagaagcaagagagtgcctctatgtggagccagatgaaggaacatccgagaagggcgtgtattggtacaggaacaagtattga

SEQ ID NO: 12 - DNA, 1101 bp, Glycine max; identical to SEQ ID NO: 9

SEQ ID NO: 13 - DNA, 1101 bp, Glycine max
cagaagaagcctctctcaagggttccaaacacaaagccaccattcactgttggccaactcaagaaagccattccaccgcactgctttcagcgttccctcctcacttcattgtcctatgttgtttatgacctttcattggctttcattttctacattgccaccacctacttccacctcctccctcaccccttttccctcattgcatggccaatctattgggttctccaaggttgcattcttactggcgtgtgggtgattgctcacgagtgtggtcaccatgccttcagcaagtacccatgggttgatgatgttgtgggtttgaccgttcactcagcacttttagtcccttatttctcatggaaaataagccatcgccgccaccactccaacacgggttcccttgaccgtgatgaagtgtttgtcccaaaaccaaaatccaaagttgcatggtacaccaagtacctgaacaaccctctaggaagggctgcttctcttctcatcacactcacaatagggtggcctttgtatttagccttcaatgtctctggcagaccctatgatggttttgctagccactaccacccttatgctcccatatattcaaatcgtgagaggcttttgatctatgtctctgatgttgctttgttttctgtgacttacttgctctaccgtgttgcaactatgaaagggttggtttggctgctatgtgtttatggggtgccattgctcattgtgaacggttttcttgtgaccatcacatatctgcagcacacacactatgccttgcctcactatgattcatcagaatgggattggctgaggggtgctttggcaactatggacagagattatgggattctgaacaaggtgtttcaccacataactgatactcatgtggctcaccatcttttctctacaatgccacattaccatgcaacggaggcaaccaatgcaatgaagccaatattgggtgagtactaccgatttgatgacacaccattttacaaggcactgtggagagaagcaagagagtgcctctatgtggagccagatgaaggaacatccgagaagggcgtgtattggtacaggaacaagtattga

SEQ ID NO: 14 - DNA, 39 bp, Artificial Sequence
  Description of Artificial Sequence: Synthetic oligonucleotide
agccatcgccgccatcactccaacacaggttcccttgac

SEQ ID NO: 15 - DNA, 43 bp, Artificial Sequence
  Description of Artificial Sequence: Synthetic oligonucleotide
tctaccgtgttgcaaccctgaaagggttggtttggctgctatg

SEQ ID NO: 16 - DNA, 41 bp, Artificial Sequence
  Description of Artificial Sequence: Synthetic oligonucleotide
gccttgcctcattacgattcatcagaatgggactggctgaa

SEQ ID NO: 17 - DNA, 41 bp, Artificial Sequence
  Description of Artificial Sequence: Synthetic oligonucleotide
ctgtgacttactctctctaccgtgttgcaaccctgaaaggg

SEQ ID NO: 18 - DNA, 39 bp, Artificial Sequence
  Description of Artificial Sequence: Synthetic oligonucleotide
agccatcgccgccaccactccaacacgggttcccttgac

SEQ ID NO: 19 - DNA, 41 bp, Artificial Sequence
  Description of Artificial Sequence: Synthetic oligonucleotide
ctgtgacttacttgctctaccgtgttgcaactatgaaaggg

SEQ ID NO: 20 - DNA, 36 bp, Artificial Sequence
  Description of Artificial Sequence: Synthetic oligonucleotide
ttcaatgtctctggcagaccctatgatggttttgct

SEQ ID NO: 21 - DNA, 24 bp, Artificial Sequence
  Description of Artificial Sequence: Synthetic primer
gtaatatgggctcagaggaatggt

SEQ ID NO: 22 - DNA, 23 bp, Artificial Sequence
  Description of Artificial Sequence: Synthetic primer
atggagaagaacattggaattgc

SEQ ID NO: 23 - DNA, 23 bp, Artificial Sequence
  Description of Artificial Sequence: Synthetic probe
ccatggcccggtaccatctggtc

SEQ ID NO: 24 - protein, 7 aa, Artificial Sequence
  Description of Artificial Sequence: Synthetic peptide
QSSDLSR

SEQ ID NO: 25 - protein, 7 aa, Artificial Sequence
  Description of Artificial Sequence: Synthetic peptide
RKDALVA

SEQ ID NO: 26 - protein, 7 aa, Artificial Sequence
  Description of Artificial Sequence: Synthetic peptide
RSADLTR

SEQ ID NO: 27 - protein, 7 aa, Artificial Sequence
  Description of Artificial Sequence: Synthetic peptide
RSDDLTR

SEQ ID NO: 28 - protein, 7 aa, Artificial Sequence
  Description of Artificial Sequence: Synthetic peptide
RSDAMSQ

SEQ ID NO: 29 - protein, 7 aa, Artificial Sequence
  Description of Artificial Sequence: Synthetic peptide
RNASRTR

SEQ ID NO: 30 - protein, 7 aa, Artificial Sequence
  Description of Artificial Sequence: Synthetic peptide
DRSNLSR

SEQ ID NO: 31 - protein, 7 aa, Artificial Sequence
  Description of Artificial Sequence: Synthetic peptide
HKWLRNQ

SEQ ID NO: 32 - protein, 7 aa, Artificial Sequence
  Description of Artificial Sequence: Synthetic peptide
DSSDRKK

SEQ ID NO: 33 - protein, 7 aa, Artificial Sequence
  Description of Artificial Sequence: Synthetic peptide
LRHHLTR

SEQ ID NO: 34 - protein, 7 aa, Artificial Sequence
  Description of Artificial Sequence: Synthetic peptide
QSGTRKT

SEQ ID NO: 35 - protein, 7 aa, Artificial Sequence
  Description of Artificial Sequence: Synthetic peptide
QNAHRKT

SEQ ID NO: 36 - protein, 7 aa, Artificial Sequence
  Description of Artificial Sequence: Synthetic peptide
QSGDLTR

SEQ ID NO: 37 - protein, 7 aa, Artificial Sequence
  Description of Artificial Sequence: Synthetic peptide
QTSTLSK

SEQ ID NO: 38 - protein, 7 aa, Artificial Sequence
  Description of Artificial Sequence: Synthetic peptide
TSGSLSR

SEQ ID NO: 39 - protein, 7 aa, Artificial Sequence
  Description of Artificial Sequence: Synthetic peptide
RSDHLTQ

SEQ ID NO: 40 - protein, 7 aa, Artificial Sequence
  Description of Artificial Sequence: Synthetic peptide
RSDVLSE

SEQ ID NO: 41 - protein, 7 aa, Artificial Sequence
  Description of Artificial Sequence: Synthetic peptide
RSADLSR

SEQ ID NO: 42 - protein, 7 aa, Artificial Sequence
  Description of Artificial Sequence: Synthetic peptide
RTDALRG

SEQ ID NO: 43 - protein, 7 aa, Artificial Sequence
  Description of Artificial Sequence: Synthetic peptide
HRSARKR

SEQ ID NO: 44 - protein, 7 aa, Artificial Sequence
  Description of Artificial Sequence: Synthetic peptide
DRSHLTR

SEQ ID NO: 45 - protein, 7 aa, Artificial Sequence
  Description of Artificial Sequence: Synthetic peptide
QSGNLHV

SEQ ID NO: 46 - protein, 7 aa, Artificial Sequence
  Description of Artificial Sequence: Synthetic peptide
RSDHLSA

SEQ ID NO: 47 - protein, 7 aa, Artificial Sequence
  Description of Artificial Sequence: Synthetic peptide
RSNLLVA

SEQ ID NO: 48 - protein, 7 aa, Artificial Sequence
  Description of Artificial Sequence: Synthetic peptide
QSGALAR

SEQ ID NO: 49 - protein, 7 aa, Artificial Sequence
  Description of Artificial Sequence: Synthetic peptide
DRSALAR

SEQ ID NO: 50 - protein, 7 aa, Artificial Sequence
  Description of Artificial Sequence: Synthetic peptide
QSSNLAR

SEQ ID NO: 51 - protein, 7 aa, Artificial Sequence
  Description of Artificial Sequence: Synthetic peptide
QSSDLRR

SEQ ID NO: 52 - protein, 7 aa, Artificial Sequence
  Description of Artificial Sequence: Synthetic peptide
RSDTLSE

SEQ ID NO: 53 - protein, 7 aa, Artificial Sequence
  Description of Artificial Sequence: Synthetic peptide
QSGHLSR

SEQ ID NO: 54 - protein, 7 aa, Artificial Sequence
  Description of Artificial Sequence: Synthetic peptide
RSDVLST

SEQ ID NO: 55 - protein, 7 aa, Artificial Sequence
  Description of Artificial Sequence: Synthetic peptide
QNAHRIK

SEQ ID NO: 56 - protein, 7 aa, Artificial Sequence
  Description of Artificial Sequence: Synthetic peptide
RSDNLSQ

SEQ ID NO: 57 - protein, 7 aa, Artificial Sequence
  Description of Artificial Sequence: Synthetic peptide
ASNDRKK

SEQ ID NO: 58 - protein, 7 aa, Artificial Sequence
  Description of Artificial Sequence: Synthetic peptide
RSDNLST

SEQ ID NO: 59 - protein, 7 aa, Artificial Sequence
  Description of Artificial Sequence: Synthetic peptide
MRQHLLN

SEQ ID NO: 60 - protein, 7 aa, Artificial Sequence
  Description of Artificial Sequence: Synthetic peptide
RSDNLAR

SEQ ID NO: 61 - protein, 7 aa, Artificial Sequence
  Description of Artificial Sequence: Synthetic peptide
QKKDRSY

SEQ ID NO: 62 - protein, 7 aa, Artificial Sequence
  Description of Artificial Sequence: Synthetic peptide
RSDHLSR

SEQ ID NO: 63 - protein, 7 aa, Artificial Sequence
  Description of Artificial Sequence: Synthetic peptide
DRSNRKT

SEQ ID NO: 64 - protein, 7 aa, Artificial Sequence
  Description of Artificial Sequence: Synthetic peptide
RSDTLSA

SEQ ID NO: 65 - protein, 7 aa, Artificial Sequence
  Description of Artificial Sequence: Synthetic peptide
DKSTRTK

SEQ ID NO: 66 - protein, 7 aa, Artificial Sequence
  Description of Artificial Sequence: Synthetic peptide
TSGSLTR

SEQ ID NO: 67 - protein, 7 aa, Artificial Sequence
  Description of Artificial Sequence: Synthetic peptide
RSDSLSA

SEQ ID NO: 68 - protein, 7 aa, Artificial Sequence
  Description of Artificial Sequence: Synthetic peptide
RSDALAR

SEQ ID NO: 69 - protein, 7 aa, Artificial Sequence
  Description of Artificial Sequence: Synthetic peptide
RRDILHQ

SEQ ID NO: 70 - protein, 7 aa, Artificial Sequence
  Description of Artificial Sequence: Synthetic peptide
QRTHLKA

SEQ ID NO: 71 - protein, 7 aa, Artificial Sequence
  Description of Artificial Sequence: Synthetic peptide
ARSTRTN

SEQ ID NO: 72 - protein, 7 aa, Artificial Sequence
  Description of Artificial Sequence: Synthetic peptide
QSGNLAR

SEQ ID NO: 73 - protein, 7 aa, Artificial Sequence
  Description of Artificial Sequence: Synthetic peptide
WRISLAA

SEQ ID NO: 74 - protein, 7 aa, Artificial Sequence
  Description of Artificial Sequence: Synthetic peptide
WKESLGA

SEQ ID NO: 75 - protein, 7 aa, Artificial Sequence
  Description of Artificial Sequence: Synthetic peptide
HRKSLSR

SEQ ID NO: 76 - protein, 7 aa, Artificial Sequence
  Description of Artificial Sequence: Synthetic peptide
YHWYLKK

SEQ ID NO: 77 - protein, 7 aa, Artificial Sequence
  Description of Artificial Sequence: Synthetic peptide
TSGHLSR

SEQ ID NO: 78 - protein, 7 aa, Artificial Sequence
  Description of Artificial Sequence: Synthetic peptide
TSGNLTR

SEQ ID NO: 79 - protein, 7 aa, Artificial Sequence
  Description of Artificial Sequence: Synthetic peptide
WWTSRAL

SEQ ID NO: 80 - DNA, 23 bp, Artificial Sequence
  Description of Artificial Sequence: Synthetic primer
cacgagtgtggtcaccatgcctt

SEQ ID NO: 81 - DNA, 26 bp, Artificial Sequence
  Description of Artificial Sequence: Synthetic primer
tgagtgtgacgagaagagaaacagcc

SEQ ID NO: 82 - DNA, 30 bp, Artificial Sequence
  Description of Artificial Sequence: Synthetic probe
agcaagtaccaatgggttgatgatgttgtg

SEQ ID NO: 83 - DNA, 24 bp, Artificial Sequence
  Description of Artificial Sequence: Synthetic primer
tgcaagccactaccacccttatgc

SEQ ID NO: 84 - DNA, 26 bp, Artificial Sequence
  Description of Artificial Sequence: Synthetic primer
ggcaaagtgtgtgtgctgcaaatatg

SEQ ID NO: 85 - DNA, 34 bp, Artificial Sequence
  Description of Artificial Sequence: Synthetic probe
ctaaccgtgagaggcttctgatctatgtctctga

SEQ ID NO: 86 - DNA, 26 bp, Artificial Sequence
  Description of Artificial Sequence: Synthetic primer
tgagtgtgatgagaagagaagcagcc

SEQ ID NO: 87 - DNA, 30 bp, Artificial Sequence
  Description of Artificial Sequence: Synthetic probe
agcaagtacccatgggttgatgatgttatg

SEQ ID NO: 88 - DNA, 26 bp, Artificial Sequence
  Description of Artificial Sequence: Synthetic primer
ttggtttggctgctatgtgtttatgg

SEQ ID NO: 89 - DNA, 28 bp, Artificial Sequence
  Description of Artificial Sequence: Synthetic primer
tgtggcattgtagagaagagatggtgag

SEQ ID NO: 90 - DNA, 32 bp, Artificial Sequence
  Description of Artificial Sequence: Synthetic probe
agggagctttggcaactatggacagagattat

SEQ ID NO: 91 - DNA, 26 bp, Artificial Sequence
  Description of Artificial Sequence: Synthetic primer
agccttcaatgtctctggcagaccct

SEQ ID NO: 92 - DNA, 26 bp, Artificial Sequence
  Description of Artificial Sequence: Synthetic primer
ggcatagtgtgtgtgctgcagatatg

SEQ ID NO: 93 - DNA, 34 bp, Artificial Sequence
  Description of Artificial Sequence: Synthetic probe
caaatcgtgagaggcttttgatctatgtctctga

SEQ ID NO: 94-118 - skipped (25 entries)

SEQ ID NO: 119 - DNA, 62 bp, Artificial Sequence
  Description of Artificial Sequence: Synthetic oligonucleotide
ttactctctctaccgtgttgcaaccctgaaatttcagggttgcaacacggtagagagagtaa

SEQ ID NO: 120 - DNA, 58 bp, Artificial Sequence
  Description of Artificial Sequence: Synthetic oligonucleotide
ttactctctctaccgtgttgcaaccctgatcagggttgcaacacggtagagagagtaa

SEQ ID NO: 121 - DNA, 57 bp, Artificial Sequence
  Description of Artificial Sequence: Synthetic oligonucleotide
ttactctctctaccgtgttgcaaccctgaaagggttgcaacacggtagagagagtaa

SEQ ID NO: 122 - DNA, 54 bp, Artificial Sequence
  Description of Artificial Sequence: Synthetic oligonucleotide
ttactctctctaccgtgttgcaaccctgaggttgcaacacggtagagagagtaa

SEQ ID NO: 123 - DNA, 30 bp, Artificial Sequence
  Description of Artificial Sequence: Synthetic oligonucleotide
ttactctctctaccgtgttgcaaccctgaa

SEQ ID NO: 124 - DNA, 60 bp, Artificial Sequence
  Description of Artificial Sequence: Synthetic oligonucleotide
ttactctctctaccgtgttgcaaccctgatttcagggttgcaacacggtagagagagtaa

SEQ ID NO: 125 - DNA, 59 bp, Artificial Sequence
  Description of Artificial Sequence: Synthetic oligonucleotide
ttactctctctaccgtgttgcaaccctgattcagggttgcaacacggtagagagagtaa

SEQ ID NO: 126 - DNA, 58 bp, Artificial Sequence
  Description of Artificial Sequence: Synthetic oligonucleotide
ttactctctctaccgtgttgcaaccctattcagggttgcaacacggtagagagagtaa

SEQ ID NO: 127 - DNA, 59 bp, Artificial Sequence; identical to SEQ ID NO: 125
  Description of Artificial Sequence: Synthetic oligonucleotide

SEQ ID NO: 128 - DNA, 59 bp, Artificial Sequence
  Description of Artificial Sequence: Synthetic oligonucleotide
ttactctctctaccgtgttgcaaccctgaatcagggttgcaacacggtagagagagtaa

SEQ ID NO: 129 - DNA, 57 bp, Artificial Sequence; identical to SEQ ID NO: 121
  Description of Artificial Sequence: Synthetic oligonucleotide

SEQ ID NO: 130 - DNA, 59 bp, Artificial Sequence
  Description of Artificial Sequence: Synthetic oligonucleotide
ttactctctctaccgtgttgcaaccctctttcagggttgcaacacggtagagagagtaa